European Patent Application EP 4 509 595 A1, published February 19, 2025. Title: Nucleated cell death induction method and using low temperature treatment. Applicant: INDUSTRY-UNIVERSITY COOPERATION FOUNDATION HANYANG UNIVERSITY. Application KR 10-2022-0045251, filed April 12, 2022. The sequence listing filed with the application follows.

SEQUENCE LISTING (4 sequences)

SEQ ID NO: 1 - DNA, 21 bp, synthetic construct
  source 1..21: mol_type = other DNA
gtcaaaagccactgtgtcctg

SEQ ID NO: 2 - DNA, 22 bp, synthetic construct
  source 1..22: mol_type = other DNA
gatttgcaaccagagacaactg

SEQ ID NO: 3 - DNA, 19 bp, synthetic construct
  source 1..19: mol_type = other DNA
gaaggtgaaggtcggagtc

SEQ ID NO: 4 - DNA, 20 bp, synthetic construct
  source 1..20: mol_type = other DNA
gacaagcttcccgttctcag